European Patent Specification EP 3 052 121 B1, published February 22, 2023. Title: Wnt compositions and methods for purification. Applicant: Jill Helms Girija Dhamdhere. The sequence listing filed with the application follows.

SEQUENCE LISTING (2 sequences)

SEQ ID NO: 1 - protein, 352 aa, Homo sapiens
MAPLGYFLLLCSLKQALGSYPIWWSLAVGPQYSSLGSQPILCASIPGLVPKQLRFCRNYVEIMPSVAEGIKIGIQECQHQFRGRRWNCTTVHDSLAIFGPVLDKATRESAFVHAIASAGVAFAVTRSCAEGTAAICGCSSRHQGSPGKGWKWGGCSEDIEFGGMVSREFADARENRPDARSAMNRHNNEAGRQAIASHMHLKCKCHGLSGSCEVKTCWWSQPDFRAIGDFLKDKYDSASEMVVEKHRESRGWVETLRPRYTYFKVPTERDLVYYEASPNFCEPNPETGSFGTRDRTCNVSSHGIDGCDLLCCGRGHNARAERRREKCRCVFHWCCYVSCQECTRVYDVHTCK

SEQ ID NO: 2 - DNA, 2826 bp, Homo sapiens
atggccccactcggatacttcttactcctctgcagcctgaagcaggctctgggcagctacccgatctggtggtcgctggctgttgggccacagtattcctccctgggctcgcagcccatcctgtgtgccagcatcccgggcctggtccccaagcagctccgcttctgcaggaactacgtggagatcatgcccagcgtggccgagggcatcaagattggcatccaggagtgccagcaccagttccgcggccgccggtggaactgcaccaccgtccacgacagcctggccatcttcgggcccgtgctggacaaagctaccagggagtcggcctttgtccacgccattgcctcagccggtgtggcctttgcagtgacacgctcatgtgcagaaggcacggccgccatctgtggctgcagcagccgccaccagggctcaccaggcaagggctggaagtggggtggctgtagcgaggacatcgagtttggtgggatggtgtctcgggagttcgccgacgcccgggagaaccggccagatgcccgctcagccatgaaccgccacaacaacgaggctgggcgccaggccatcgccagccacatgcacctcaagtgcaagtgccacgggctgtcgggcagctgcgaggtgaagacatgctggtggtcgcaacccgacttccgcgccatcggtgacttcctcaaggacaagtacgacagcgcctcggagatggtggtggagaagcaccgggagtcccgcggctgggtggagaccctgcggccgcgctacacctacttcaaggtgcccacggagcgcgacctggtctactacgaggcctcgcccaacttctgcgagcccaaccctgagacgggctccttcggcacgcgcgaccgcacctgcaacgtcagctcgcacggcatcgacggctgcgacctgctgtgctgcggccgcggccacaacgcgcgagcggagcggcgccgggagaagtgccgctgcgtgttccactggtgctgctacgtcagctgccaggagtgcacgcgcgtctacgacgtgcacacctgcaagtaggcaccggccgcggctccccctggacggggcgggccctgcctgagggtgggcttttccctgggtggagcaggactcccacctaaacggggcagtactcctccctgggggcgggactcctccctgggggtggggctcctacctgggggcagaactcctacctgaaggcagggctcctccctggagctagtgtctcctctctggtggctgggctgctcctgaatgaggcggagctccaggatggggaggggctctgcgttggcttctccctggggacggggctcccctggacagaggcggggctacagattgggcggggcttctcttgggtgggacagggcttctcctgcgggggcgaggcccctcccagtaagggcgtggctctgggtgggcggggcactaggtaggcttctacctgcaggcggggctcctcctgaaggaggcggggctctaggatggggcacggctctggggtaggctgctccctgagggcggagcgcctccttaggagtggggttttatggtggatgaggcttcttcctggatggggcagagcttctcctgaccagggcaaggccccttccacgggggctgtggctctgggtgggcgtggcctgcataggctccttcctgtgggtggggcttctctgggaccaggctccaatggggcggggcttctctccgcgggtgggactcttccctgggaaccgccctcctgattaaggcgtggcttctgcaggaatcccggctccagagcaggaaattcagcccaccagccacctcatccccaaccccctgtaaggttccatccacccctgcgtcgagctgggaaggttccatgaagcgagtcgggtccccaacccgtgcccctgggatccgagggcccctctccaagcgcctggctttggaatgctccaggcgcgccgacgcctgtgccaccccttcctcagcctggggtttgaccacccacctgaccaggggccctacctggggaaagcctgaagggcctcccagcccccaaccccaagaccaagcttagtcctgggagaggacagggacttcgcagaggcaagcgaccgaggccctcccaaagaggcccgccctgcccgggctcccacaccgtcaggtactcctgccagggaactggcctgctgcgccccaggccccgcccgtctctgctctgctcagctgcgcccccttctttgcagctgcccagcccctcctccctgccctcgggtctccccacctgcactccatccagctacaggagagatagaagcctctcgtcccgtccctccctttcctccgcctgtccacagccccttaagggaaaggtaggaagagaggtccagccccccaggctgcccagagctgctggtctcatttgggggcgttcgggaggtttggggggcatcaaccccccgactgtgctgctcgcgaaggtcccacagccctgagatgggccggcccccttcctggcccctcatggcgggactggagaaatggtccgctttcctggagccaatggcccggcccctcctgactcatccgcctggcccgggaatgaatggggaggccgctgaacccacccggcccatatccctggttgcctcatggccagcgcccctcagcctctgccactgtgaaccggctcccaccctcaaggtgcggggagaagaagcggccaggcggggcgccccaagagcccaaaagagggcacaccgccatcctctgcctcaaattctgcgtttttggttttaatgttatatc